European Patent Specification EP 3 421 500 B1, published March 5, 2025. Title: METHOD FOR EXPRESSING AND PREPARING POLYVALENT MULTI-SPECIFIC ANTIBODY AND IMMUNE HYBRID PROTEIN. Applicant: SHANGHAI JIAO TONG UNIVERSITY JECHO LABORATORIES, INC. JECHO BIOPHARMACEUTICALS CO.,LTD. The sequence listing filed with the application follows.

SEQUENCE LISTING (4 sequences)

SEQ ID NO: 1 - DNA, 40 bp, Artificial Sequence
  Sig-Her-For
aaaaagcttatgggttggagctgcatcatcttgttcctcg

SEQ ID NO: 2 - DNA, 43 bp, Artificial Sequence
  Her-HC-OL-Nn-Rev
gccaccacctgatccgcctccgcctgacttcccggggctcagg

SEQ ID NO: 3 - DNA, 54 bp, Artificial Sequence
  Nn-OL-HerHC-For
ggcggatctggtggtggcggatcttattgtttaagctatgaaacggaaatattg

SEQ ID NO: 4 - DNA, 63 bp, Artificial Sequence
  Nn-Rev-BamHI
aaaggatcctcagtggtggtggtggtggtggtggtggtggtgattcggcaaattatcaacccg